European Patent Application EP 4 624 582 A1, published October 1, 2025. Title: MICROORGANISMS FOR PRODUCING PURINE NUCLEOTIDES AND PROCESS FOR PRODUCING PURINE NUCLEOTIDES USING THE SAME. Applicant: CJ CheilJedang Corporation. The sequence listing filed with the application follows.

SEQUENCE LISTING (63 sequences)

SEQ ID NO: 1 - DNA, 35 bp, synthetic construct
  source 1..35: mol_type = other DNA
gtacccggggatcctgaaatcatcagcgttggccc

SEQ ID NO: 2 - DNA, 38 bp, synthetic construct
  source 1..38: mol_type = other DNA
gaactcgtggtgatggtgactatatattcccttcgtcg

SEQ ID NO: 3 - DNA, 36 bp, synthetic construct
  source 1..36: mol_type = other DNA
ggaatatatagtcaccatcaccacgagttccttcag

SEQ ID NO: 4 - DNA, 35 bp, synthetic construct
  source 1..35: mol_type = other DNA
attctgggtagtcatgagtgtttcctttcgttggg

SEQ ID NO: 5 - DNA, 37 bp, synthetic construct
  source 1..37: mol_type = other DNA
cgaaaggaaacactcatgactacccagaattcttccg

SEQ ID NO: 6 - DNA, 35 bp, synthetic construct
  source 1..35: mol_type = other DNA
gcaggtcgactctagggaagactgcagagttgagc

SEQ ID NO: 7 - DNA, 35 bp, synthetic construct
  source 1..35: mol_type = other DNA
acccggggatcctctagagtgccgttacctcccgc

SEQ ID NO: 8 - DNA, 36 bp, synthetic construct
  source 1..36: mol_type = other DNA
tggagtgcgtagcgtgcgaaatgactcctttctaaa

SEQ ID NO: 9 - DNA, 36 bp, synthetic construct
  source 1..36: mol_type = other DNA
tttagaaaggagtcatttcgcacgctacgcactcca

SEQ ID NO: 10 - DNA, 36 bp, synthetic construct
  source 1..36: mol_type = other DNA
aagcttgcatgcctgcagcgtcaccgcgcggagata

SEQ ID NO: 11 - DNA, 25 bp, synthetic construct
  source 1..25: mol_type = other DNA
gaaatgactcctttctaaaaagggg

SEQ ID NO: 12 - DNA, 39 bp, synthetic construct
  source 1..39: mol_type = other DNA
ttagaaaggagtcatttcgaacttgcagcaaacgtgctg

SEQ ID NO: 13 - DNA, 20 bp, synthetic construct
  source 1..20: mol_type = other DNA
ccttggtgaggcactttgtg

SEQ ID NO: 14 - DNA, 39 bp, synthetic construct
  source 1..39: mol_type = other DNA
caaagtgcctcaccaagggcacgctacgcactccatata

SEQ ID NO: 15 - DNA, 20 bp, synthetic construct
  source 1..20: mol_type = other DNA
gtcaacgcgcacttggatct

SEQ ID NO: 16 - DNA, 38 bp, synthetic construct
  source 1..38: mol_type = other DNA
aattcgagctcggtacccaggcacagccgacattacgg

SEQ ID NO: 17 - DNA, 35 bp, synthetic construct
  source 1..35: mol_type = other DNA
gtagcacatctgacgaatgtccaagtctaaggaaa

SEQ ID NO: 18 - DNA, 35 bp, synthetic construct
  source 1..35: mol_type = other DNA
ttagacttggacattcgtcagatgtgctacttgcc

SEQ ID NO: 19 - DNA, 35 bp, synthetic construct
  source 1..35: mol_type = other DNA
tgcgccattagcgtgttacttctcgcggctataga

SEQ ID NO: 20 - DNA, 35 bp, synthetic construct
  source 1..35: mol_type = other DNA
agccgcgagaagtaacacgctaatggcgcattgaa

SEQ ID NO: 21 - DNA, 35 bp, synthetic construct
  source 1..35: mol_type = other DNA
tgaattatccgcgtcttagatgccgttttctgccg

SEQ ID NO: 22 - DNA, 35 bp, synthetic construct
  source 1..35: mol_type = other DNA
gaaaacggcatctaagacgcggataattcagctgt

SEQ ID NO: 23 - DNA, 38 bp, synthetic construct
  source 1..38: mol_type = other DNA
cgactctagaggatccccgatgaagcgaacacttaaat

SEQ ID NO: 24 - DNA, 20 bp, synthetic construct
  source 1..20: mol_type = other DNA
ccagtacattgtcatgggat

SEQ ID NO: 25 - DNA, 20 bp, synthetic construct
  source 1..20: mol_type = other DNA
gattggcatatcgcaccgag

SEQ ID NO: 26 - DNA, 38 bp, synthetic construct
  source 1..38: mol_type = other DNA
tcgagctcggtacccgttgccgtatcagacatgctcag

SEQ ID NO: 27 - DNA, 38 bp, synthetic construct
  source 1..38: mol_type = other DNA
gattagcctgaaggaattgatttatctcgaccaaacag

SEQ ID NO: 28 - DNA, 38 bp, synthetic construct
  source 1..38: mol_type = other DNA
ggtcgagataaatcaattccttcaggctaatcttttcc

SEQ ID NO: 29 - DNA, 38 bp, synthetic construct
  source 1..38: mol_type = other DNA
cgatataagactccatcatatgtgtttcctttcgttgg

SEQ ID NO: 30 - DNA, 38 bp, synthetic construct
  source 1..38: mol_type = other DNA
aaaggaaacacatatgatggagtcttatatcggtagcc

SEQ ID NO: 31 - DNA, 38 bp, synthetic construct
  source 1..38: mol_type = other DNA
ctcataggtgccgaacttactcggagatttcgacctca

SEQ ID NO: 32 - DNA, 38 bp, synthetic construct
  source 1..38: mol_type = other DNA
cgaaatctccgagtaagttcggcacctatgagaatatg

SEQ ID NO: 33 - DNA, 39 bp, synthetic construct
  source 1..39: mol_type = other DNA
ctctagaggatccccggcaagtgtttcttggcgccattc

SEQ ID NO: 34 - DNA, 19 bp, synthetic construct
  source 1..19: mol_type = other DNA
gcgagggggaagaaaagta

SEQ ID NO: 35 - DNA, 18 bp, synthetic construct
  source 1..18: mol_type = other DNA
cgttgccctttttcttct

SEQ ID NO: 36 - DNA, 38 bp, synthetic construct
  source 1..38: mol_type = other DNA
aattcgagctcggtaccccatttcgtgaccattagcgt

SEQ ID NO: 37 - DNA, 35 bp, synthetic construct
  source 1..35: mol_type = other DNA
attagcctgaaggaagatcatgccaatagcgccag

SEQ ID NO: 38 - DNA, 35 bp, synthetic construct
  source 1..35: mol_type = other DNA
gctattggcatgatcttccttcaggctaatctttt

SEQ ID NO: 39 - DNA, 35 bp, synthetic construct
  source 1..35: mol_type = other DNA
attctgggtagtcatcatatgtgtttcctttcgtt

SEQ ID NO: 40 - DNA, 35 bp, synthetic construct
  source 1..35: mol_type = other DNA
aaggaaacacatatgatgactacccagaattcttc

SEQ ID NO: 41 - DNA, 35 bp, synthetic construct
  source 1..35: mol_type = other DNA
ctttgtacttggtgaccaagagtcaggatgccgaa

SEQ ID NO: 42 - DNA, 35 bp, synthetic construct
  source 1..35: mol_type = other DNA
catcctgactcttggtcaccaagtacaaagagact

SEQ ID NO: 43 - DNA, 38 bp, synthetic construct
  source 1..38: mol_type = other DNA
cgactctagaggatccccggttaccgcgcattaggact

SEQ ID NO: 44 - DNA, 20 bp, synthetic construct
  source 1..20: mol_type = other DNA
taatcccccagctcaccggc

SEQ ID NO: 45 - DNA, 20 bp, synthetic construct
  source 1..20: mol_type = other DNA
tttggatgccgaggtcgtag

SEQ ID NO: 46 - protein, 433 aa, Corynebacterium stationis
MTTQNSSDAQYQEMRDLDPEVYAAINGEIARQRDTLEMIASENFVPRAVLQAQGSVLTNKYAEGYPGRRYYGGCEHVDIVEDLARDRAKALFGAEFANVQPHSGAQANAAVLASLINPGDKILGLSLAHGGHLTHGMKLNFSGKLYEVAAYEVDAETNRIDMDKLREQAIAEKPQVIIAGWSAYPRTLDFEAYRSIADEVGAYLWTDMAHFAGLVAADLYPNPVPHSDIVSTTVHKTLGGPRSGMILAKQDYAKKLNSAVFPGQQGGPLMHVVAAKAIAMKVAASEEFRDRQVRTLEGAKILAERLTTPEAKAAGVDVLTGGTDVHLVLADLRNSEMDGQQAEDLLHEVGITVNRNAVPNDPRPPMVTSGLRIGTSALATRGLDAEAFTEVADIIGTALTDGKNADTQKLRARVDKLAEQFPLYEGLEDWKIV

SEQ ID NO: 47 - DNA, 1302 bp, Corynebacterium stationis
  source 1..1302: mol_type = genomic DNA
atgactacccagaattcttccgatgctcagtaccaggaaatgcgtgacttagacccagaggtctatgcagcaattaacggtgaaattgctcgtcagcgcgataccctggagatgattgcgtcggagaactttgttcctcgtgcagtcttgcaggcacagggttccgtccttaccaacaagtacgcagagggctacccaggtcgccgctactacggtggatgtgagcacgtcgatatcgtcgaagatctggcgcgtgaccgcgctaaggctctgttcggcgctgagtttgccaatgtacagccacactccggtgcacaggcaaacgctgccgtccttgcttctcttatcaacccaggcgataagatcttgggcctttctttggctcacggtggtcacctgacccacggcatgaagctgaacttctccggcaagctctacgaagtagctgcctacgaagtcgatgcagaaaccaaccgtatcgacatggacaagctgcgtgagcaggctattgcagaaaagccacaggtcatcatcgctggctggtctgcatacccacgcactctggattttgaagcataccgttccatcgcggatgaagtgggggcttacctgtggaccgatatggcacactttgctggtctcgttgccgctgatctgtacccaaatccagttccacactctgacattgtttccaccaccgtgcacaagaccctgggcggtcctcgctccggcatgatcctggctaagcaggactacgctaagaagctcaactctgcagtcttcccaggccagcagggtggccctttgatgcatgtggttgcagcgaaggcaattgccatgaaggttgctgcttccgaagaattccgtgaccgtcaggtccgtactctggaaggcgcgaagattcttgctgagcgcttgaccactcctgaggcaaaggcagcaggcgttgacgttctcactggcggcaccgacgtgcacttggttcttgcggacctgcgcaattctgagatggatggccagcaggcagaagacctcctgcacgaggtcggcatcaccgttaaccgcaacgcggttccaaacgatccacgtccaccaatggtgacctctggtctgcgtatcggtacttccgctctggctacccgcggcctggatgcagaagcattcaccgaggtggcagacatcatcggcaccgcgcttaccgatggcaagaacgccgatacccagaagctgcgcgcacgcgtggacaagcttgctgagcagttcccactctacgagggcttggaagactggaagatcgtctaa

SEQ ID NO: 48 - protein, 470 aa, Corynebacterium stationis
VTISVIDIFSVGVGPSSSHTVGPMRAAKTFMESLPHAPAKVHTELRGSLSATGKGHATDRAVILGLAGWAPLTVPIDAKPLAGSFIPSEGTVEGPAGSVQYSIAFNNKPVPEHPNCLIFSAWDENGEEIATNMEYFSVGGGFVLSRAELDAQLQATHEVPAGMAAAQNNDNAIPYDFSTGDQLLELCDEHDMTIWEIVAANEAVIHREDGGLAKVNAHLDLVWDVMRECVTDGIATKGILPGGLQVNRRAPQLYSQLLEHQDDTASGFSAMEWVNLYALAVNEQNAAGGRVVTAPTNGACGIIPAVLHYARDFLPDFTRETARRFLLTAGAIGMIIKQNASISGAEVGCQGEVGSASSMAAAGLAEILGSSPAQIENAAEIALEHNLGLTCDPVGGLVQIPCIERNAIGAVKSINSARLARMGEGTHYVTLDNAVQTMAETGRDMLTKYKETSIGGLAKTLGLSVSQVEC

SEQ ID NO: 49 - DNA, 1413 bp, Corynebacterium stationis
  source 1..1413: mol_type = genomic DNA
gtgaccattagcgtcattgacatcttttcagtaggcgtggggccttcgtcctcccacaccgttggccccatgcgtgcagcgaaaacctttatggaatctttgccgcatgctcctgccaaagtacatactgagctgcgtggttcactctcagccacgggtaaaggccacgccaccgaccgcgccgtcattttaggccttgccggatgggcgccacttaccgtacctattgacgctaagccgcttgccggcagttttatcccttctgaaggcacagtcgaaggccccgccggcagcgtgcagtattccattgcgttcaacaacaagccggtgcctgagcacccgaactgtttgatatttagcgcctgggatgaaaatggtgaagaaatcgctaccaatatggagtacttctccgtgggcggcggctttgttctctcacgtgcagagctcgatgcgcagctgcaagccacccacgaagttccggcgggtatggcggctgcgcaaaataatgacaacgcaatcccctatgacttcagcaccggtgatcagctcctagagttgtgcgatgagcacgacatgacaatctgggaaatcgtcgctgccaatgaagcagttattcaccgtgaagatggtgggctggccaaggtcaacgcgcacttggatctggtgtgggatgtcatgcgtgagtgtgttactgatggcattgctaccaaggggattttgcccggtggtctgcaggttaatcgtcgtgctccgcaactttatagtcaattgcttgaacaccaagatgatactgcgtcaggcttttctgccatggagtgggtcaacctctatgcactagccgtcaacgagcaaaatgctgccggtggccgcgtggtcactgctccaactaacggtgcctgcggaatcattcccgcggtcttgcactatgcacgagacttcctccccgatttcactcgtgagacagcccggcgttttctgctcaccgctggcgctattggcatgatcatcaagcagaatgcttctatctctggcgctgaggttggctgccaaggagaagtcggctcggcatcgtcaatggctgctgccgggttggctgagattttaggctcgagtccagcacagatcgaaaatgcggcagaaatagcactcgagcacaatctcggtctaacctgcgatccggtcggcggcttggtgcagattccgtgcatcgagcgcaatgcgattggcgcagtaaagtctattaactccgcacgccttgcccgcatgggtgaaggcacgcattacgtcaccctcgataatgctgtgcagacaatggccgagaccggccgagacatgctcaccaagtacaaagagacttcgatcggtggcttggctaagaccctgggactatctgtctcccaggtggagtgctaa

SEQ ID NO: 50 - protein, 361 aa, Corynebacterium stationis
MTATTNHLTENSHAHGYDHYQRMAFFTDTSVCIGCKACEVACKEWNRNPVEGYNLTGNSYDNTGALGANTWRHVAFIEQDNERITKAREEGAKLVSLGMPTIGTSPVDAAPNPASADTTPPDTDTFRWLMSSDVCKHCTNAGCLDVCPTGALFRTEFGTVVVQDDVCNGCGTCVAGCPFGVIERREDGGVSLKANHVEAQEVPEHAGINVFKKLKQLRPQGPDHVPGETMPIKNIGVAQKCTMCYDRLKVGEQPACSKTCPTESIQFGTYENMLAAAQARVAELHRQGQTEARLYGANNEDGVGGTGSIFLLLDSPEVYGLPPDPRVPTADLPAMAKTFAKAVGAMGVAVAASFLVDRGGT

SEQ ID NO: 51 - DNA, 1086 bp, Corynebacterium stationis
  source 1..1086: mol_type = genomic DNA
atgacggctacgaccaatcacctaacagaaaattcgcacgcgcacggctacgaccattaccagcgcatggcctttttcaccgatacttcggtgtgcattggctgtaaggcttgcgaggtggcctgtaaggagtggaaccgcaacccggttgagggctataacctgacgggtaattcctacgacaacaccggcgcgctgggcgcgaatacctggcgacacgtagcatttattgagcaagacaacgagcgcatcaccaaagcgcgtgaagaaggtgccaagctggtctcgctgggcatgccgacgattggcacttcgcctgtcgatgcagccccgaatcctgcctccgccgataccacgccgccggatactgatactttccgttggctgatgtcttctgatgtctgcaagcactgcaccaacgctggctgcctggatgtgtgcccaaccggtgctttatttcgcaccgaatttggcaccgtcgtggtccaagatgatgtctgcaatggctgcggcacctgcgttgccgggtgcccgttcggtgttattgagcgccgtgaagacggcggtgtttcgctaaaagccaaccacgtcgaagcccaagaagtccctgaacacgcgggcattaacgtgtttaagaagctcaaacagctgcgcccgcaaggaccggatcacgtcccgggtgagaccatgccgattaaaaatattggcgtggctcaaaagtgcaccatgtgctacgaccgcctgaaagtcggcgagcagccagcgtgttccaagacatgcccgacggagtccatccagttcggcacctatgagaatatgctggccgctgcgcaagcgcgcgtggctgagctacaccgtcaaggccagactgaggcacgactgtacggcgcaaataacgaagacggcgtcggcggaacgggctccatcttcttgctgctggattccccggaagtctacggtcttccaccagatccgcgtgtgccgactgcagatttgcccgcaatggcgaagactttcgccaaggccgttggcgccatgggcgttgccgtggcagcgtcctttttagttgatagaggagggacctag

SEQ ID NO: 52 - protein, 923 aa, Corynebacterium stationis
LGTSFGRGGATQPLQDMANADCILIQGSNMAECHPVGFQWVVEAKKRGARVIHVDPRYTRTSAFANRHVAIRGGTDVVLLGALIKYMIDNDLYFHDYVVNYTNASSIISPDFRDTEDLDGLFSGYNPETGKYITDSWQYVQKPEGAWWNIERDETLQDPNTVFQILKRHYSRYTPEIVEETCGISQEDFHYLAESIAQNSNPERTTVFAYALGFTQQTLGVQFIRAAAILQLLMGNVGRPGSGIMALRGHASIQGSTDIPTLFNNLPGYLPMPHADHGDWKGFLDAIAKEDQKGFWGLRENYAVSLMKSYWGENATKDNDWGWNYMPRINGAHSTYETLMGMLDGIVEGYIVFGQNPAVAQSNGGMQRRGLASLKWLVVRDFQEIETASFWYDSPEIKTGELKTEDIGTEVFLLPAATHVEKAGTFTQTQRMLQWRFQATNPPGDAKSDLWFFYQMGKRIREKLAGSTDPMDAPLLAIDWNYEETEHGEPDPEDVLREINGYYLDGPKKGQLLPGFTEMKPDGTTSGGCWIYSGVFKDNINQSARKVSGASQNEVALEWGWVWPSNRRMLYNRASAAPDGTPWSERKKYIWWDAEAGRWTGDDVPDFPVNLDPSYRAPVDATGPAALDGTDAFIMQADGRGWLFVPKGLSDGPLPTHYEPHESPARNILYSQQQSPTRLTIKRPDNLSKPMAGEPGSEVYPVVFSTYRLTEMYTSGAMSRRLPYLAELQPDLFVEVDPVLAQKRGLENGGWATIISPRGVIEARVLVTERMESMTINGKDFHQIGLPFHYGQSSSSPVTGDGANDLLGLTLEPNVFIQNSKVGACEIKAGRRPRGKARLEMLKEYQRRAGLTLDTGNELIDPDAQQLEATSTIDLFIPNGVDKETVETSTSEPGAADGSAHHGSAMGEVPNSEPKDTEGGEKQ

SEQ ID NO: 53 - DNA, 2772 bp, Corynebacterium stationis
  source 1..2772: mol_type = genomic DNA
ttgggaacctcgtttggccgcggtggcgcaactcagccactgcaggatatggcaaatgccgactgcatcctgattcagggctcgaatatggccgagtgccatcctgtgggtttccagtgggtagtcgaagctaaaaagcgcggggcgcgcgtaattcacgtggatcctcgctatacccgtacctcggcgtttgcgaaccggcacgtagcgatccgtggcggcaccgatgtggtgcttcttggcgcacttatcaagtacatgatcgacaatgatctgtattttcacgactatgtggtcaattacacgaacgcgtcgtcgatcatttctcccgacttccgggacacggaagacctagacggcctcttttctggctacaacccagaaaccggtaagtacatcacggactcgtggcagtacgtgcaaaagcccgaaggtgcgtggtggaatatcgagcgtgatgagactttgcaggacccgaatacggtcttccagattctcaagcgccactattcccgctataccccggaaatcgtggaagagacctgcggtatctcccaggaggacttccattatctagcggagtcgattgcacagaactccaatccagagcgcactacagtctttgcctatgctttgggctttacgcagcaaaccttaggcgtgcagttcattcgtgccgcggccatcttgcaactgctgatgggcaacgtgggccgcccgggctcaggcatcatggcgctgcgtggacacgcttccattcagggctcgacagatatcccgacgctgtttaataacttgccgggttacttgccgatgcctcatgccgaccatggcgactggaaaggattcttggacgcgattgccaaggaagaccagaagggtttctggggtctgcgtgaaaactatgccgtgagcttgatgaagtcctattggggcgagaatgccaccaaggacaatgactggggctggaactacatgccgcgcatcaacggtgcgcactccacctatgaaaccttgatgggcatgctcgacggcatcgtcgaaggctatatcgtcttcggacaaaacccagcggtcgctcaatccaacggcggcatgcaacgccgcggattggcgtctttgaagtggttggttgttcgtgacttccaggaaattgagacagcgtcattctggtacgactcaccagagatcaagactggtgaactcaagaccgaagatattggcaccgaggtcttccttcttcctgcagcaacgcacgtagaaaaggccggtacctttacccaaacccagcgcatgctgcagtggcgtttccaggccacaaatccaccaggcgatgccaagagcgatctgtggttcttctaccagatgggcaagcgcattcgcgaaaagcttgctggttctactgatccgatggacgcgccattgttggccatcgactggaactacgaggaaaccgaacacggcgagccagatcccgaagacgtgctgcgcgaaatcaacggctactatctggatggcccgaagaaggggcagctgctgcctggctttacagagatgaagcctgatggcacgacgtctggtggctgctggatctactccggcgtgttcaaggacaacatcaaccagtccgcgcgcaaagtttcaggcgcttcgcaaaatgaggttgcgctggaatggggctgggtatggccatcgaatcgccgcatgctgtacaaccgtgcgtcagctgcgccagacggcacgccatggtcggagcgcaagaagtacatttggtgggacgctgaggccggccgctggacgggcgacgacgtaccggacttcccagtcaacttggatccgtcataccgcgcgcctgtcgatgccacaggtcctgcagcccttgacggcaccgatgcgtttatcatgcaggcagatggtcgtggttggttgttcgtacccaaaggactttccgatggacccctgccaacccactatgaaccgcacgagtcgccggcacgcaatattttgtacagccagcagcagtcgccgacacgcttgaccatcaagcgtccggataacttgtcgaagcccatggctggtgagcccggctcagaggtctaccccgtggttttctccacgtaccgtttgacggagatgtacacctcgggtgcgatgagccgccgactgccttatttggcagagttgcagccagatttgttcgttgaggtcgatccggttctagcacaaaagcgcggcttggaaaacggtggctgggcaaccatcatttcgccgcgtggcgtgattgaggctcgcgtgctggtgaccgaacgcatggaatctatgaccatcaatggcaaggacttccaccagattggtctgcctttccactacggtcagtccagctcctcgccagttactggtgacggtgccaatgaccttctgggtctaactttggagccgaatgtgttcattcaaaactccaaggttggtgcatgtgaaattaaggccggccgacgcccacgcggcaaggcgcggttagagatgctcaaggaataccagcgccgtgccggattgacgttggacaccggtaacgagctcatcgatcccgatgcacagcagctcgaagctacctccacgatcgacttatttattccgaatggcgtagacaaagagacggtggagacatcgacaagcgagcctggcgccgcagatggttctgcgcatcatggctcagcgatgggggaagtcccaaattctgaaccaaaagatacggagggaggcgaaaagcaatga

SEQ ID NO: 54 - protein, 188 aa, Corynebacterium stationis
MSKLSPLNWPVVRQVKRGDLFGRDKSTQSAKSENLHGRTVEADKVVQSVCPYCAVGCSQRVYVKDDRVVHIEGDSDSPISRGRLCPKGAASEQLVNSATRLTKIKYRAPHATEWQDLDLETAMDMIADRFIASRRNQWQDFDEKGRVLNRTMGVAGLGGATLDNEENYIIKKLFTAAGAVQVENQARI

SEQ ID NO: 55 - DNA, 567 bp, Corynebacterium stationis
  source 1..567: mol_type = genomic DNA
atgtcgaagttaagtccgctgaattggccggttgtgcgccaggtgaagcgcggcgatctgtttggtcgagataaatcaacccagtctgccaaatcggagaacctgcacgggcgcactgtagaggccgacaaagtagttcaatcggtctgcccttactgcgctgtgggctgctcgcagcgggtatatgtcaaagatgaccgcgtcgttcatattgaaggtgactcggactcgcctatttcgcgcggacgtttgtgcccgaaaggcgctgcctctgagcagctggtgaactctgcgacgcgtttgaccaagattaaataccgcgcgcctcatgcaaccgagtggcaagacctagatctcgaaaccgcaatggatatgattgcggaccgttttattgcctcccgccgcaatcagtggcaggactttgatgaaaaaggccgtgttttaaaccgcaccatgggtgtggcaggacttggtggcgccaccttggataatgaggaaaactacattatcaagaagctgtttactgcagctggtgccgtacaagtcgaaaaccaagcacgcatatga

SEQ ID NO: 56 - protein, 952 aa, Corynebacterium stationis
MDFIARHLGPDATESKDMLARVGYDSVEALVTSAIPQSISITDALNMPQALSETDAQAKLRAYADKNVVLKSFYGQGYSDTITPAVIRRGLVEDAGWYTAYTPYQPEISQGRLESLLNFQTMVQDLTGLPIANASLLDEASAVAEAVGLMSRAVKKGRRVLLDARLHPQVLTVAAERARAIDLEVEIADLSNGVVGEDLVGAVVAYTGTEGDIFDPRAVIEEIHGRGGLVSVAADLLSLLLLEGPGSFGADIVIGSSQRFGVPLFFGGPHAAFMAVTDKLKRQMPGRLVGVSVDSEGRPAYRLALQTREQHIRRERATSNICTAQALLANVAAMYAVYHGPEGLKEIANHVHSLAASFAGAVTTQGLKITSSEFFDTVTVAGVDAASIKFSLEKAGYLVRTIGEDKVSVSFGESATQGDVTVLADAFGAAAVDNADFPLPEALTRTTEVLTHEIFNSIHSETQMMRYLRKLGDKDLALDRTMIPLGSCTMKLNPTAAMEPITWPEFANVHPYSPEYATQGWRELIEELEGWLAELTGYAKVSIQPNAGSQGELAGLLAIRRYHVANGDTNRDIVLIPASAHGTNAASATLANLRVVVVKTAEDGSIDLEDLDAKIAKHGQNMAGIMITYPSTHGVFDPEVREVCDKIHAAGGQVYIDGANMNALTGWAQPGKFGGDVSHLNLHKTFTIPHGGGGPGVGPIGVAEHLIPFLPTDAAADELDPANPTPVEQGVPITASQFGSAGVLPITWAYIAMTGGEGLTSATAHAILGANYLARELSDSFPILFTGNEGLVAHECILDLRALTDASGVTAADVAKRLIDFGFHAPTLAFPVAGTLMVEPTESEDIAELDRFIEAMRTIRAEIQEIIDGKIAYEDSVIRHAPYTAPSVSSDDWEYSFSREKAAWPVPSLRLNKYFPPVRRLDEAYGDRNLVCSCPPPEAFDFDADTDSTEEA

SEQ ID NO: 57 - DNA, 2859 bp, Corynebacterium stationis
  source 1..2859: mol_type = genomic DNA
atggatttcattgcccgccaccttgggccagatgccacagaatctaaggacatgctggcgcgtgtgggttatgacagcgtagaagcgcttgtcacctcagcaatcccccagtccattagcatcacggatgcgcttaatatgccgcaggcattgagtgagaccgacgcacaagccaagcttcgcgcttacgctgataaaaatgtcgtgctgaagtctttctacggccagggctactcagacaccatcacccctgctgttattcgccgcggtttggtagaagacgctggttggtacaccgcttataccccataccagccagaaatttcccagggtcgccttgagtcgctgctgaacttccagaccatggttcaagacctcaccggcttgcctattgcgaatgcttctttgctggatgaggcatcggcagttgctgaggccgtgggtttgatgtctcgtgcggtcaagaagggccgccgcgtactgctcgacgcccgtttgcacccacaggttctcaccgtggcggcggagcgtgcccgagcaattgacctcgaagttgagattgctgacttgagcaacggcgtggttggcgaagacctcgtcggcgcagtagttgcctacaccggtacggagggcgatatttttgacccacgtgctgttatcgaagaaatccatggccgcggcggacttgtttccgtcgcggctgacttgttgtccttgctgcttctggaaggcccaggctcgttcggtgcagacattgtcattggttcctcccaacgctttggtgtgccgctcttctttggtggcccacacgctgctttcatggcagtaactgacaagctaaagcgtcagatgccaggccgtttggtcggcgtatcggtcgattctgagggccgtcctgcttaccgcttggcgctgcagactcgtgaacagcacatccgccgtgaacgcgcgacgtcaaatatttgtaccgcgcaggcacttctggccaacgtggctgccatgtacgccgtctaccacggtccagaaggcttgaaggagattgctaaccacgtgcactccttggctgcttcctttgccggtgcagttactactcagggtctgaagattacttcctcggagttcttcgacaccgttaccgttgccggcgttgatgccgcatccattaagttcagcttggaaaaggccggatacctggtgcgcaccattggcgaggataaggtttctgtctccttcggtgagtccgcaacccaaggcgatgttactgtcttggcggacgcctttggtgccgctgcagtagataatgcagatttcccactgcctgaagcactcacccgcaccaccgaggtgctcacccacgaaatctttaactccattcactccgaaacccagatgatgcgttacctgcgcaagctcggtgataaggatctggctctagatcgcaccatgattcctttgggctcatgcaccatgaagctcaacccaaccgcagccatggaaccgatcacctggccagaattcgccaatgttcacccttactcccctgaatacgcaacccagggctggcgtgagctcattgaagagttggaaggctggttggctgagctgaccggctacgccaaggtttctatccaaccaaacgctggttcccagggcgagctagctggtcttttggctatccgccgctaccacgtcgcaaatggtgacaccaaccgcgatatcgtgttgattcctgcgtccgcgcacggcaccaacgctgcctccgcgaccctggcaaatctgcgcgttgttgtggttaagaccgccgaagacggctccatcgatctggaagatctcgatgcgaagatcgccaagcatggtcagaacatggccggaatcatgatcacctacccatccactcacggcgtctttgacccagaggttcgtgaagtctgcgacaagatccatgccgctggcggccaggtctacattgatggcgcaaacatgaatgctttgactggttgggctcagccgggcaagttcggtggcgatgtctcgcacttgaacctgcacaagactttcaccattccgcacggcggtggcggcccaggtgttggaccaattggtgtcgctgagcacctcattccattcctgccaacggatgctgcagctgatgagctggatcctgctaacccaaccccagtagaacagggcgttccaattactgcttcgcagtttggttccgctggtgttctgccgattacctgggcatacatcgcaatgaccggtggcgagggtctaacctccgctactgcacacgccatcttgggtgctaactaccttgcgcgcgaactctccgattccttcccaattctgttcaccggtaatgaaggtcttgttgcgcacgagtgcattttggatctgcgcgcgctaaccgatgcctcaggcgttactgcagcagacgttgccaagcgtttgatcgactttggcttccacgctcctaccctcgcattcccagtggctggcaccttgatggtggaacctactgagtctgaggatattgctgaactggatcgtttcattgaagcaatgcgcaccatccgtgcggagattcaggaaatcatcgatggcaagatcgcatatgaagattcggtcatccgccacgcaccttacaccgcaccgtcagtctcaagcgatgattgggagtactcctttagccgtgaaaaggccgcatggccagttccttcactgcgtttgaacaagtacttcccaccggtacgccgcctggatgaagcttacggcgaccgcaacctggtgtgctcctgcccaccgccagaggcattcgacttcgatgccgacaccgattccaccgaggaggcttaa

SEQ ID NO: 58 - protein, 367 aa, Corynebacterium stationis
MSELRQSPLHAEHEKLGASFTAFGPWNMPLKYGKELDEHHAVRNAVGMFDLSHMGEIWVNGPDAAAFLSYALISNMETVKNGKAKYSMIVAEDGGIIDDLISYRFSDTKFLVVPNAGNTDVVWEAFNQRIEGFDVELNNESLDVAMIALQGPNAAKVLVEQVAEESKEEVENLPYYAATMAKVADVDTIVARTGYTGEDGFELMIYNADATKLWQLFIDQDGVTPCGLASRDSLRLEAGMPLYGNELSRDITPVEAGMGVAFKKKTADFVGAEVLRQRLEEGPKQVIKALTSSERRAARTGAEIYAGEQLVGTVTSGQPSPTLGHPIALALVDTAANLEEGAEVEVDIRGKRYPFTVTKTPFYSREK

SEQ ID NO: 59 - DNA, 1104 bp, Corynebacterium stationis
  source 1..1104: mol_type = genomic DNA
atgtcagaactacgccagtccccactgcacgcagagcacgaaaagctcggcgcatcctttaccgcttttggcccttggaatatgccactaaagtacggcaaggagctcgatgagcaccacgcagtgcgtaatgcagtcggcatgtttgacctctcgcacatgggtgagatttgggtcaacggcccagacgccgctgcatttttgtcctatgcgctgatctccaacatggagaccgtgaaaaatggcaaggcgaagtactccatgattgttgctgaagacggcggcatcatcgatgacctaatttcctaccgtttctccgataccaagttcttggtagtgccaaacgctggcaacactgatgtggtttgggaagcttttaatcagcgcattgaaggcttcgatgtagaactcaacaatgagtccttggatgttgcgatgattgccctgcagggccccaatgctgccaaggttctagttgaacaggttgctgaagagtccaaggaagaagtagaaaaccttccttactatgccgcaaccatggccaaagtcgcagacgttgacaccatcgtcgcgcgcaccggctacaccggcgaagacggcttcgagctgatgatctacaacgccgatgcgaccaagctctggcagcttttcatcgaccaagatggtgttactccatgcggtttagcttcacgcgattccttgcgcttggaagctggcatgcctttgtacggcaatgagctttcccgcgatatcacccctgtcgaggcaggcatgggtgtggcgtttaagaagaagaccgctgacttcgtcggcgccgaggtcctgcgtcaacgcttggaagaaggccctaagcaagttatcaaggctttgacctcctctgagcgccgtgcagcgcgcaccggtgctgaaatctatgccggcgagcagttggtaggcaccgtaacttcgggtcagccatcgccgacgctgggacaccctattgccctggcactggtagatactgcagcaaacctcgaagaaggcgcagaagtagaagtggatattcgcggcaagcgttaccccttcaccgttaccaagacgcctttctatagccgcgagaagtaa

SEQ ID NO: 60 - protein, 129 aa, Corynebacterium stationis
MANLPAEFTYSEDHEWINAAQDAIVGKTVRIGITSVAADRLGEVVFAELPAVGDSVTAGETCGEVESTKSVSDLYSPVTGTVTAVNETVHDDYEIINNDPFGEGWLFEVEVEELGEVMTADEYAAENGI

SEQ ID NO: 61 - DNA, 390 bp, Corynebacterium stationis
  source 1..390: mol_type = genomic DNA
atggctaacctacctgcagaatttacttactccgaagaccacgagtggattaacgccgctcaggacgcaatcgttggcaaaactgttcgcatcggcatcacttctgttgccgcagaccgtcttggtgaggttgtcttcgctgagcttccagcagttggcgatagcgtcactgcaggtgaaacctgtggtgaggttgaatccaccaagtccgtttctgacctgtacagccctgtcaccggtaccgtgaccgctgtgaacgagacagtgcacgatgattatgaaatcatcaacaatgatcctttcggtgaaggttggctgtttgaggtcgaggttgaagaactcggcgaggttatgaccgctgatgaatacgcggcagaaaacggcatctaa

SEQ ID NO: 62 - protein, 422 aa, Corynebacterium stationis
LESYIGSPLTSNAVRVLMLGGGELAKGLVGAFQNLGLEVHVVDRYEGSPAQQVAHFSYTADIDDEKAVLDLVEHIKPAYVVPEIEGVADEALHALHDDSAVTVVPTARACELTSDRKKLREVAESLGLPTTAYKVVETFDALKEAVNELGLPCIIKPDVATSGRGHVLVKDEDQLKDAWDNVRRGKKNSWVVAERFVDFDYEVIIMAVRSIDPETGKLATWFSEPIGYEHARGNLVDCWQPKTMSQRAFENARSVAARISNELGGRGIFAVELFVAGDDIYFSSVTPRPSDKAMLTEATQRFSQYELHARAILGLPIDITLVSPGASSLLHATEEIDEVTYSGVEEALQVAETDVRLFGKPSAYPGRRMGLIMATADDVSEARDRAAIAASKITISAAPRLVPEPELTSEKELSPDEVEISE

SEQ ID NO: 63 - DNA, 1269 bp, Corynebacterium stationis
  source 1..1269: mol_type = genomic DNA
ttggagtcttatatcggtagccccctgacctcgaatgctgttcgggttctcatgctcggcggcggtgagctggccaaaggtttggtgggcgcgtttcagaatttgggcttggaagtccacgttgtcgaccgctatgaggggtctccagcacagcaggttgcacactttagctacaccgcagatatcgatgatgaaaaggccgtgctcgatttagttgagcacatcaagccggcttatgtcgtgccagaaatcgagggcgtagcagatgaggctttgcatgcgcttcacgatgactccgctgtcaccgttgtgcccaccgcccgggcgtgtgagcttaccagcgaccggaagaagctacgcgaagtcgcagaaagcctcggcttgccgacgaccgcgtacaaggtcgtagaaaccttcgacgctttgaaagaagcggtgaacgagctcggtttgccgtgcattattaagccggatgttgcaacctctggacgcgggcatgtgctggtcaaagacgaagaccaactcaaagacgcgtgggataatgtgcgtcgcggcaagaagaactcctgggttgtcgccgaacgctttgtggattttgactatgaagtcatcatcatggcggtgcgctcgattgacccggaaacgggcaagctggcaacgtggttctcagagccgattggttatgagcatgcgcgcggcaacctcgtggactgctggcagccaaagacgatgagccagcgtgcttttgaaaatgcacgttcggttgcagcgcgtatttctaacgaactcggcggccgcggcatcttcgcggtggagctgtttgtcgcgggcgacgatatctacttctcctcggtgaccccgcgtccttctgataaagcgatgctgaccgaagccacccaacgcttttcgcagtatgaattgcacgcgcgcgccattttgggcctgccgatcgacatcacgcttgtctcaccgggcgctagctctttgttgcacgcgaccgaagagatcgacgaagttacctactcgggcgttgaagaagccctgcaggttgcagaaaccgatgtgcgcctattcggcaagccttcggcataccctggccgacgcatggggttgatcatggccaccgccgacgatgtctccgaagcacgcgaccgcgctgcgatcgcggcatcgaagatcacgattagcgccgccccaaggttagttcctgaaccagaactaacctctgaaaaagagttatcccccgatgaggtcgaaatctccgagtaa